European Patent Specification EP 3 773 675 B1, published December 4, 2024. Title: SYSTEMS AND METHODS FOR CHARACTERIZING SURFACTANT PROTEIN D (SP-D) OLIGOMERS. Applicant: Jan Susan Rosenbaum Mark Cornell Manning Ryan R. Manning. The sequence listing filed with the application follows.

SEQUENCE LISTING (2 sequences)

SEQ ID NO: 1 - protein, 376 aa, homo sapiens
  Human SP-D polypeptide including a leader sequence. With polymorphisms at: Met 31, Thr 180, Ser  290, Ala 306.
MLLFLLSALVLLTQPLLGYLEAEMKTYSHRTMPSACTLVMCSSVESGLPGRDGRDGREGPRGEKGDPGLPGAAGQAGMPGQAGPVGPKGDNGSVGEPGPKGDTGPSGPPGPPGVPGPAGREGPLGKQGNIGPQGKPGPKGEAGPKGEVGAPGMQGSAGARGLAGPKGERGVPGERGVPGNTGAAGSAGAMGPQGSPGARGPPGLKGDKGIPGDKGAKGESGLPDVASLRQQVEALQGQVQHLQAAFSQYKKVELFPNGQSVGEKIFKTAGFVKPFTEAQLLCTQAGGQLASPRSAAENAALQQLVVAKNEAAFLSMTDSKTEGKFTYPTGESLVYSNWAPGEPNDDGGSEDCVEIFTNGKWNDRACGEKRLVVCEF

SEQ ID NO: 2 - protein, 355 aa, homo sapiens
  SP-D polypeptide of SEQ ID NO:01, without leader sequence. With polymorphisms at: Met 11, Thr 160, Ser  270, Ala 286.
AEMKTYSHRTMPSACTLVMCSSVESGLPGRDGRDGREGPRGEKGDPGLPGAAGQAGMPGQAGPVGPKGDNGSVGEPGPKGDTGPSGPPGPPGVPGPAGREGPLGKQGNIGPQGKPGPKGEAGPKGEVGAPGMQGSAGARGLAGPKGERGVPGERGVPGNTGAAGSAGAMGPQGSPGARGPPGLKGDKGIPGDKGAKGESGLPDVASLRQQVEALQGQVQHLQAAFSQYKKVELFPNGQSVGEKIFKTAGFVKPFTEAQLLCTQAGGQLASPRSAAENAALQQLVVAKNEAAFLSMTDSKTEGKFTYPTGESLVYSNWAPGEPNDDGGSEDCVEIFTNGKWNDRACGEKRLVVCEF